European Patent Application EP 4 520 836 A1, published March 12, 2025. Title: Method and kit for the enzymatic degradation of poly(allyl diglycol carbonate). Applicant: ESSILOR INTERNATIONAL. Application EP. The sequence listing filed with the application follows.

SEQUENCE LISTING (8 sequences)

SEQ ID NO: 1 - protein, 342 aa, Candida antarctica
MKLLSLTGVAGVLATCVAATPLVKRLPSGSDPAFSQPKSVLDAGLTCQGASPSSVSKPILLVPGTGTTGPQSFDSNWIPLSTQLGYTPCWISPPPFMLNDTQVNTEYMVNAITALYAGSGNNKLPVLTWSQGGLVAQWGLTFFPSIRSKVDRLMAFAPDYKGTVLAGPLDALAVSAPSVWQQTTGSALTTALRNAGGLTQIVPTTNLYSATDEIVQPQVSNSPLDSSYLFNGKNVQAQAVCGPLFVIDHAGSLTSQFSYVVGRSALRSTTGQARSADYGITDCNPLPANDLTPEQKVAAAALLAPAAAAIVAGPKQNCEPDLMPYARPFAVGKRTCSGIVTP

SEQ ID NO: 2 - protein, 565 aa, Sus scrofa
MWLLPLVLTSLASSATWAGQPASPPVVDTAQGRVLGKYVSLEGLAQPVAVFLGVPFAKPPLGSLRFAPPQPAEPWSFVKNTTSYPPMCCQDPVVEQMTSDLFTNGKERLTLEFSEDCLYLNIYTPADLTKRGRLPVMVWIHGGGLVLGGAPMYDGVVLAAHENVVVVAIQYRLGIWGFFSTGDEHSRGNWGHLDQVAALHWVQENIANFGGDPGSVTIFGESAGGESVSVLVLSPLAKNLFHAISESGVALTVALVRKDMKAAAKQIAVLAGCKTTTSAVFVHCLRQKSEDELLDLTLKMKFLTLDFHGDQRESHPFLPTVVDGVLLPKMPEEILAEKDFNTVPYIVGINKQEFGWLLPTMMGFPLSEGKLDQKTATSLLWKSYPIANIPEELTPVATDKYLGGTDDPVKKKDLFLDLMGDVVFGVPSVTVARQHRDAGAPTYMYEFQYRPSFSSDKKPKTVIGDHGDEIFSVFGFPLLKGDAPEEEVSLSKTVMKFWANFARSGNPNGEGLPHWPMYDQEEGYLQIGVNTQAAKRLKGEEVAFWNDLLSKEAAKKPPKIKHAEL

SEQ ID NO: 3 - protein, 764 aa, Sus scrofa
MDLRTMTQSLVTLAEDNMAFFSGQGPGETARRLSGVFAGIREQALGLEPALGRLLSVAHLFDLDAETPANGYRSLVHTARCCLAHLLHKSRYVASNRRSIFFRTSHNLAELEAYLAALTQLRALAYYAQRLLAINRPGKLFFEGDEGITADFLREYVTLHKGCFYGRCLGFQFTPAIRPFLQTISIGLVSFGEHYKRNETGLSVTASSLFTSGRFAIDPELRGAEFERIIQNLDVHFWKAFWNITEIEVLSSLANMASATVRVSRLLSLPPKAFEMPLTADPKLTVTISPPLAHTGPGPVLVRLISYDLREGQDSEELSSLVRSEGPRGLELRPRPQQAPRSRSLVVHIHGGGFVAQTSKSHEPYLKSWAQELGVPILSIDYSLAPEAPFPRALEECFYAYCWAVKHCGLLGSTGERICLAGDSAGGNLCFTVSLRAAAYGVRVPDGIMAAYPATMLQSAASPSRLLSLMDPLLPLSVLSKCVSAYAGGEMEDHSDSDQKALGMMGLVRRDTALLFRDLRLGASSWLNSFLELSGHKSRPNLVPTEEPMRRSVSEAALAQPEGPLGTDSLKYLTLHDLSLSSETQDTPELSLSAETLGPTTPSAVNFLFRPEDAPEEAEARDDISTKEEKVYSVRAAFPEGFHPRRSSQGAIQMPLYSAPIVKNPFMSPLLAPDSMLQTLPPVHIVACALDPMLDDSVMFARRLRSLGQPVTLHVVEDLPHGFLSLAALCRETRQAAALCVDRIRFILNPPGPATPAGPTTPPV

SEQ ID NO: 4 - protein, 282 aa, unidentified
MRKFTLGCLSATALVALSVSATAAPLPDTPGAPFPSVSSFDNDGPYAVTSQSEGPNCRVYRPRTLGQGGVRHPIILWGNGTGTGPTTYSGLLTHWASHGFVVAAAETSNAGTGREMLACLDYLVQESNRTYGTYVGVLNTGRVGTSGHSQGGGGSIMAGQDDRVKATAPIQPYTIGLGHDSSSQRNQRGPMFLMSGGADTIAIPYLNAQPVFTRANVPIFWGERRYVSHFEPVGNGGEYRGPSTAWFRYQLMDDQSARSTFYGRLCRLCTSLLWSVERKGIE

SEQ ID NO: 5 - protein, 301 aa, unidentified
MAVMTPRRERSSLLSRALQVTAAAATALVTAVSLAAPAHAANPYERGPNPTDALLEASSGPFSVSEENVSRLSASGFGGGTIYYPRENNTYGAVAISPGYTGTEASIAWLGERIASHGFVVITIDTITTLDQPDSRAEQLNAALNHMINRASSTVRSRIDSSRLAVMGHSMGGGGTLRLASQRPDLKAAIPLTPWHLNKNWSSVTVPTLIIGADLDTIAPVATHAKPFYNSLPSSISKAYLELDGATHFAPNIPNKIIGKYSVAWLKRFVDNDTRYTQFLCPGPRDGLFGEVEEYRSTCPF

SEQ ID NO: 6 - protein, 482 aa, unidentified
MTELTVQTRCGALKGTAGHGVRTWKSIPYAKPPVGELRFKAPEPPVPWDGVKNADSFGPVCPQPADLLSMSFSGDVPPQSEDCLYLNVFAPDSEGGKRPVMVWIHGGAFFLGAGSEPTYDASALAADGDVIVVTLNYRLGPFGFLHLFSIDDTYPGNIGMLDQIAALRWVKDNISAFGGDPDNVTVFGESAGGMSIASLMAMPDAKGLFHKAILESGASQTMTADVAKEITTAFIQEAGTDQLQELSVNDILKTADKLRNTIDQSIFHLLFQPAIDPATLPAEPAKAIADGAAEGIPMIIGTNRDEAYLFFTPDTDIHSEKKQQEYLLYHLGENSAKLAADLYPHSLTGQIDMMTDLKFWRPAVAFAQEQSQYAPVWMYRFDWHGETPPFHKAVHALELPFVFGNFDSLKKTLKEPLSEDVKQLSKLIQSAWIAFAKTGKPDTDQLHWPQYETGSRETIIFNTSVSTESDPDSAKRRILFQA

SEQ ID NO: 7 - protein, 293 aa, unidentified
MSASSLKFPIVLVHGLLGFDKIGGIYPYFYGIKEALEKAGAKVYIATLSALNSNELRGEQLLEFVRKVQAETGAAKVNLIGHSQGPLACRYVAATHPELIASVTSVNGVNHGSEVADLVRLALTPGRLPESIANAAMSAFGQLLSALAGSPRLPQSGIEALEALTSEGVAAFNKKYPQGLPAEWGGEGKELVNGVYYYSWSGIIDYNPLHQGANNLDPLHVAMLAFSILFTNERFQNDGLVGRYSSHLGKVIGSDYSMDHVDAINQLAGVVANNTDPVQLFVEHVARLKSKGL

SEQ ID NO: 8 - protein, 299 aa, unidentified
MKKLVALLIVGLFVSISLTGLGLAGGTAPYKCDTRYPVVLAHGMGASTKILGIVDYWYGIEDALKAEGASVYFTSVNAMGSTVDKAADFKQQFMEILAVTGAPKANIIGHSHGTLYTRYAISNLGLAPYVASYTSLAGPHRGSAVASLIMYDLPDWLLAAGGDVLNFVYTFIFGDTNPDSLQNALDLCPDYMVNTFNPNTPNIPGIYYQSWAAKAKTSCPSVILEPTWLIMLIEEGANDGLVSVESAKWGNFRGVEDAAWYSAGCDHLNIVGQLFGVTPGFDAPQFFVDIVEDLKGRGY